European Patent Application EP 4 239 068 A1, published September 6, 2023. Title: Antibody specifically binding to nucleocapsid protein of Severe Acute Respiratory Syndrome Coronavirus 2 or its fragment and use of the same. Applicant: TOYOBO CO., LTD NATIONAL UNIVERSITY CORPORATION UNIVERSITY OF TOYAMA. The sequence listing filed with the application follows.

SEQUENCE LISTING (152 sequences)

SEQ ID NO: 1 - protein, 172 aa, Homo sapiens
MSDNGPQNQRNAPRITFGGPSDSTGSNQNGERSGARSKQRRPQGLPNNTASWFTALTQHGKEDLKFPRGQGVPINTNSSPDDQIGYYRRATRRIRGGDGKMKDLSPRWYFYYLGTGPEAGLPYGANKDGIIWVATEGALNTPKDHIGTRNPANNAAIVLQLPQGTTLPKGFY

SEQ ID NO: 2 - protein, 173 aa, Homo sapiens
TKKSAAEASKKPRQKRTATKAYNVTQAFGRRGPEQTQGNFGDQELIRQGTDYKHWPQIAQFAPSASAFFGMSRIGMEVTPSGTWLTYTAAIKLDDKDPNFKDQVILLNKHIDAYKTFPPTEPKKDKKKKADETQALPQRQKKQQTVTLLPAADLDDFSKQLQQSMSSADSTQA

SEQ ID NO: 3 - protein, 8 aa, Guinea pig
GFTFDDYG

SEQ ID NO: 4 - protein, 8 aa, Guinea pig
GFTFSDFW

SEQ ID NO: 5 - protein, 8 aa, Guinea pig
GFTFNNYW

SEQ ID NO: 6 - protein, 8 aa, Guinea pig
GFTFDDFG

SEQ ID NO: 7 - protein, 8 aa, Guinea pig
GFTFSNYY

SEQ ID NO: 8 - protein, 8 aa, Guinea pig
GFTFSDYW

SEQ ID NO: 9 - protein, 8 aa, Guinea pig
GFSLTSYS

SEQ ID NO: 10 - protein, 8 aa, Guinea pig
GFTFSDYT

SEQ ID NO: 11 - protein, 10 aa, Guinea pig
GFSITTNGYT

SEQ ID NO: 12 - protein, 8 aa, Guinea pig
ISYSGGRT

SEQ ID NO: 13 - protein, 8 aa, Guinea pig
INYDGDRT

SEQ ID NO: 14 - protein, 8 aa, Guinea pig
INGDSTKI

SEQ ID NO: 15 - protein, 8 aa, Guinea pig
IDYSGGTT

SEQ ID NO: 16 - protein, 8 aa, Guinea pig
ISYSGGST

SEQ ID NO: 17 - protein, 8 aa, Guinea pig
ISGDSNYI

SEQ ID NO: 18 - protein, 8 aa, Guinea pig
IHPDGGST

SEQ ID NO: 19 - protein, 8 aa, Guinea pig
ISPDGGGT

SEQ ID NO: 20 - protein, 8 aa, Guinea pig
ISPSGGST

SEQ ID NO: 21 - protein, 8 aa, Guinea pig
ISYSGGNT

SEQ ID NO: 22 - protein, 8 aa, Guinea pig
IWYDGTKM

SEQ ID NO: 23 - protein, 8 aa, Guinea pig
ISGDTNYI

SEQ ID NO: 24 - protein, 7 aa, Guinea pig
IWYDADT

SEQ ID NO: 25 - protein, 7 aa, Guinea pig
IWSGGRI

SEQ ID NO: 26 - protein, 15 aa, Guinea pig
ARDGGSYYSPINFQF

SEQ ID NO: 27 - protein, 15 aa, Guinea pig
SRDGGSYHSPISCQY

SEQ ID NO: 28 - protein, 15 aa, Guinea pig
ARDGGSYSSPINFQY

SEQ ID NO: 29 - protein, 15 aa, Guinea pig
SRDGGSYSSPINFQY

SEQ ID NO: 30 - protein, 15 aa, Guinea pig
ARDGGSVTSPIYFQV

SEQ ID NO: 31 - protein, 15 aa, Guinea pig
ARDGGSVKSPIYFQY

SEQ ID NO: 32 - protein, 8 aa, Guinea pig
ATNYNFQY

SEQ ID NO: 33 - protein, 8 aa, Guinea pig
ATSGPMDV

SEQ ID NO: 34 - protein, 19 aa, Guinea pig
ARSIIAEIPTIFTFPPFDV

SEQ ID NO: 35 - protein, 11 aa, Guinea pig
ARLWSGYALDI

SEQ ID NO: 36 - protein, 13 aa, Guinea pig
AKYYDYDYTGFDV

SEQ ID NO: 37 - protein, 14 aa, Guinea pig
VSPLLVVHGPFFQY

SEQ ID NO: 38 - protein, 14 aa, Guinea pig
VSPLLVYHGPFFQY

SEQ ID NO: 39 - protein, 14 aa, Guinea pig
VKPLLVLHGPFFQS

SEQ ID NO: 40 - protein, 10 aa, Guinea pig
VSPSGAGLDV

SEQ ID NO: 41 - protein, 9 aa, Guinea pig
SPSAVGFDV

SEQ ID NO: 42 - protein, 7 aa, Guinea pig
SEYKHYN

SEQ ID NO: 43 - protein, 7 aa, Guinea pig
SEHRSYY

SEQ ID NO: 44 - protein, 7 aa, Guinea pig
SDYSHYS

SEQ ID NO: 45 - protein, 7 aa, Guinea pig
SQGINKW

SEQ ID NO: 46 - protein, 7 aa, Guinea pig
SGHSSYY

SEQ ID NO: 47 - protein, 7 aa, Guinea pig
SEHSSYY

SEQ ID NO: 48 - protein, 7 aa, Guinea pig
SDHSSYY

SEQ ID NO: 49 - protein, 13 aa, Guinea pig
SQSLFYSGKNKDL

SEQ ID NO: 50 - protein, 6 aa, Guinea pig
NIGGKT

SEQ ID NO: 51 - protein, 7 aa, Guinea pig
LKSDGSH

SEQ ID NO: 52 - protein, 7 aa, Guinea pig
VKSDGSH

SEQ ID NO: 53 - protein, 7 aa, Guinea pig
IESDGSH

SEQ ID NO: 54 - protein, 7 aa, Guinea pig
VKSDGSL

SEQ ID NO: 55 - protein, 7 aa, Guinea pig
LNSYGSH

SEQ ID NO: 56 - protein, 7 aa, Guinea pig
LNSKGSH

SEQ ID NO: 57 - protein, 7 aa, Guinea pig
IESKGSH

SEQ ID NO: 58 - protein, 8 aa, Guinea pig
VGTSDIVG

SEQ ID NO: 59 - protein, 10 aa, Guinea pig
GVSYSGGHNI

SEQ ID NO: 60 - protein, 10 aa, Guinea pig
GVSFSGGHGV

SEQ ID NO: 61 - protein, 10 aa, Guinea pig
GVSYSGGHNV

SEQ ID NO: 62 - protein, 10 aa, Guinea pig
GVSVSGGHNL

SEQ ID NO: 63 - protein, 10 aa, Guinea pig
GVSLKGGHNL

SEQ ID NO: 64 - protein, 11 aa, Guinea pig
GADYSGASSYV

SEQ ID NO: 65 - protein, 13 aa, Guinea pig
GANHNIGESYGYV

SEQ ID NO: 66 - protein, 9 aa, Guinea pig
GVGYNNKYV

SEQ ID NO: 67 - protein, 9 aa, Guinea pig
GVGYSGGYV

SEQ ID NO: 68 - protein, 9 aa, Guinea pig
GVSYSGGYV

SEQ ID NO: 69 - protein, 9 aa, Guinea pig
GVKYSGGVV

SEQ ID NO: 70 - protein, 9 aa, Guinea pig
GVSYSGGYY

SEQ ID NO: 71 - protein, 9 aa, Guinea pig
QYDSTPPLT

SEQ ID NO: 72 - protein, 9 aa, Guinea pig
QVWDSYTYV

SEQ ID NO: 73 - protein, 8 aa, Guinea pig
QFINGPLT

SEQ ID NO: 74 - protein, 8 aa, Guinea pig
GFIFSNYF

SEQ ID NO: 75 - protein, 8 aa, Guinea pig
GFTFNTYT

SEQ ID NO: 76 - protein, 8 aa, Guinea pig
GFTFSNYY

SEQ ID NO: 77 - protein, 8 aa, Guinea pig
GLSLTNYT

SEQ ID NO: 78 - protein, 8 aa, Guinea pig
GFSFSNSW

SEQ ID NO: 79 - protein, 8 aa, Guinea pig
GFTFSNYW

SEQ ID NO: 80 - protein, 8 aa, Guinea pig
GFTFRNHW

SEQ ID NO: 81 - protein, 8 aa, Guinea pig
GFTFSNHW

SEQ ID NO: 82 - protein, 8 aa, Guinea pig
GFFFSNSW

SEQ ID NO: 83 - protein, 8 aa, Guinea pig
GFTFDDYG

SEQ ID NO: 84 - protein, 6 aa, Guinea pig
KLSERY

SEQ ID NO: 85 - protein, 8 aa, Guinea pig
ISGDSTYI

SEQ ID NO: 86 - protein, 8 aa, Guinea pig
IGNSGSKT

SEQ ID NO: 87 - protein, 8 aa, Guinea pig
ISGDGSNI

SEQ ID NO: 88 - protein, 8 aa, Guinea pig
ISGDSSNI

SEQ ID NO: 89 - protein, 8 aa, Guinea pig
IKGDSSII

SEQ ID NO: 90 - protein, 8 aa, Guinea pig
INPDDGSP

SEQ ID NO: 91 - protein, 8 aa, Guinea pig
IKGDSSIT

SEQ ID NO: 92 - protein, 8 aa, Guinea pig
INSDGSNT

SEQ ID NO: 93 - protein, 8 aa, Guinea pig
INTDGSST

SEQ ID NO: 94 - protein, 8 aa, Guinea pig
IKGDSRTI

SEQ ID NO: 95 - protein, 8 aa, Guinea pig
ISGASSNI

SEQ ID NO: 96 - protein, 8 aa, Guinea pig
ISGDSSNV

SEQ ID NO: 97 - protein, 8 aa, Guinea pig
IKGDSSTI

SEQ ID NO: 98 - protein, 8 aa, Guinea pig
INSDGSST

SEQ ID NO: 99 - protein, 8 aa, Guinea pig
IGYSGASI

SEQ ID NO: 100 - protein, 8 aa, Guinea pig
ISGTSSNI

SEQ ID NO: 101 - protein, 7 aa, Guinea pig
MWSDGDT

SEQ ID NO: 102 - protein, 7 aa, Guinea pig
TINWGDV

SEQ ID NO: 103 - protein, 7 aa, Guinea pig
STLGVGV

SEQ ID NO: 104 - protein, 7 aa, Guinea pig
TTLGVGV

SEQ ID NO: 105 - protein, 7 aa, Guinea pig
STTGFDV

SEQ ID NO: 106 - protein, 7 aa, Guinea pig
STLGNFL

SEQ ID NO: 107 - protein, 7 aa, Guinea pig
TITWGDV

SEQ ID NO: 108 - protein, 7 aa, Guinea pig
TIDWGNV

SEQ ID NO: 109 - protein, 19 aa, Guinea pig
ARTSRIVADLVTMGYALDF

SEQ ID NO: 110 - protein, 16 aa, Guinea pig
ARDVVKTGTTGLPFDL

SEQ ID NO: 111 - protein, 14 aa, Guinea pig
AREGVITVGTWGDV

SEQ ID NO: 112 - protein, 5 aa, Guinea pig
ATSEY

SEQ ID NO: 113 - protein, 6 aa, Guinea pig
TTATDV

SEQ ID NO: 114 - protein, 6 aa, Guinea pig
TPATDV

SEQ ID NO: 115 - protein, 10 aa, Guinea pig
SPMTIHGLDT

SEQ ID NO: 116 - protein, 5 aa, Guinea pig
GSGWV

SEQ ID NO: 117 - protein, 5 aa, Guinea pig
GSGWY

SEQ ID NO: 118 - protein, 10 aa, Guinea pig
LSSESDDARV

SEQ ID NO: 119 - protein, 6 aa, Guinea pig
KLSNQY

SEQ ID NO: 120 - protein, 6 aa, Guinea pig
KLSERY

SEQ ID NO: 121 - protein, 6 aa, Guinea pig
KLSKEY

SEQ ID NO: 122 - protein, 6 aa, Guinea pig
ALPKKY

SEQ ID NO: 123 - protein, 6 aa, Guinea pig
KLSTQY

SEQ ID NO: 124 - protein, 6 aa, Guinea pig
KLSDQY

SEQ ID NO: 125 - protein, 12 aa, Guinea pig
SESLLHSDGNTY

SEQ ID NO: 126 - protein, 12 aa, Guinea pig
SQSLLHSDGKTY

SEQ ID NO: 127 - protein, 12 aa, Guinea pig
SQSLVHSDGKTY

SEQ ID NO: 128 - protein, 12 aa, Guinea pig
SQSLLDSDGYTY

SEQ ID NO: 129 - protein, 12 aa, Guinea pig
SQSLLYSDGYTY

SEQ ID NO: 130 - protein, 12 aa, Guinea pig
SQSLLYSDGYTF

SEQ ID NO: 131 - protein, 12 aa, Guinea pig
SQSLLHSDGNTY

SEQ ID NO: 132 - protein, 12 aa, Guinea pig
SQSLLHGDGKTY

SEQ ID NO: 133 - protein, 6 aa, Guinea pig
NIGGKA

SEQ ID NO: 134 - protein, 11 aa, Guinea pig
LSRQSDDAASV

SEQ ID NO: 135 - protein, 11 aa, Guinea pig
LSSESDDAARV

SEQ ID NO: 136 - protein, 11 aa, Guinea pig
LSRESNDAAWV

SEQ ID NO: 137 - protein, 11 aa, Guinea pig
LSADSSGTYRV

SEQ ID NO: 138 - protein, 11 aa, Guinea pig
LSRQSDTAASL

SEQ ID NO: 139 - protein, 11 aa, Guinea pig
LSRQGDTAASY

SEQ ID NO: 140 - protein, 10 aa, Guinea pig
LSGESDDAWV

SEQ ID NO: 141 - protein, 9 aa, Guinea pig
LQATHDPYT

SEQ ID NO: 142 - protein, 9 aa, Guinea pig
VQTTHDPYT

SEQ ID NO: 143 - protein, 9 aa, Guinea pig
LQATHNPVS

SEQ ID NO: 144 - protein, 9 aa, Guinea pig
LQATHDPIT

SEQ ID NO: 145 - protein, 9 aa, Guinea pig
VQTSHVPLT

SEQ ID NO: 146 - protein, 9 aa, Guinea pig
VQTTHVPLT

SEQ ID NO: 147 - protein, 8 aa, Guinea pig
QTTNDPYT

SEQ ID NO: 148 - protein, 9 aa, Guinea pig
QVYDSSSFV

SEQ ID NO: 149 - protein, 8 aa, Guinea pig
WQGTDFPR

SEQ ID NO: 150 - protein, 12 aa, Homo sapiens
LLPAADLDDFSK

SEQ ID NO: 151 - protein, 9 aa, Homo sapiens
KKADETQAL

SEQ ID NO: 152 - protein, 8 aa, Homo sapiens
SAAEASKK